European Patent Specification EP 4 161 543 B1, published January 28, 2026. Title: COMPOSITIONS AND METHODS FOR INHIBITING THE PROLIFERATION OF PATHOGENIC ESCHERICHIA COLI. Applicant: iNtRON Biotechnology, Inc. The sequence listing filed with the application follows.

SEQUENCE LISTING (1 sequence)

SEQ ID NO: 1 - DNA, 40403 bp, Unknown
  Podoviridae bacteriophage
tctcacagttcaagaacctcaagtccccccataggccctctttaagtccgaccaaaggccctacccctagaccgaaggtctaaacctcaagtcactagtcgtcgactagcagccattgacccgaagtctgacccgaagtctggaccgatagggcctatatctagtggttgggacgatgggttgggactatatgttgtgtccctgagtcgctatctgtatcagcccaaagtcatcacctacagtctcactacctacagtctcactacctacagtctcactacctagttagccttcagctaacctacagtcatcgaccatcggtaaagccactacctacagtcaccgacctacagttaatagacacaatctatagacttaaggtctaagacatgttagtcaaagattatatcctcttagtcactatggggccgacgatagcttaatcaatattatttcaaattacctattgactataggtctagactatggctaatagcttccgtcaacacgacacggcaacaaccggatagtgaagacgccgggtcagaccggataagtagtcagcctgtaagacatacgaacaacaggcatctgacagaaagtagttgacaagcagtaacgaattaaagtagtatgtaccacatcaagtcaacacgattgataggcagacagaaagtgttagcttcccggaattagaagtattagtgaccgggtgttgtaacgggtctgcaccgctctttaacaatctggataaactcttaatgtgcgccgatagctagcttgctagcgatagcgactaactacagggtctttgagtctacatctgaaggccctgactgatagtcactaactataggataaacaagatggcatgatttctaaccaccagtacaacacatggtctaacccattttaaggaactacaatcatgaaactgataggcaaaggcgcgttcactaagtgctacctgaaggattgcgggaagcgtgtacttctggtctcttctgacccgataaaagagtgtatggcgcggggatggttccctgagtctccactgttccctgaagtcaagatgattgaggttggcacgtatgagatggactacatgccaccaacacgaggtctcaaggcgcatttagacgacgaccagtggcaactctatcaggtgctgcgcgattgctcctcacggtctccgtatgtaatgcgacctgctgacctgtatcccaagtggtacgagatattccaagctgcacacgacaggtccgagtctgagactgtgcgggagggcctgatggatgttctgatggcgctggacgcttgcgctaacttcgggtcagacattcagtttgagataagcccacgtaatgtacgggctgtggatggcaagctgatactggttgactgtttctttcttgtgtccaagctgcgagaggtgatgtcatcaagatgataacttatggtctctgccagcaccacgtcaccaacgcccggcttctggtcaagaccgggcagttaaaccacgatgcgactatgcgccacctgaaagcggtctatgagggacgcaagcgcatacacgacagtttgcacgctgaggataagtaaacatgtaccagataacttatagcagtgaacaggcgttctacgatggatgctacgagatgatgaagcgcggagcctgctacgtggctaatcaccatagcctgaccataacgcttacaggcgggtactgatatcttaacgagtgttaaactacaggtcatctacatggtggcctgactgattgtcacttaaccacaagaaggaaacacgtaatgaacgcacacgataaagtaatcatgaacaacctgatgtctcagcttcacgctatcatctgcgaggcgtgctacaagactgaagactcaagcgcaggcatagcaggtcagccgcgctggggagcctttgagatactggcccatgagcatggttacaagctgttaggcttagggcatttcgctgccgcctttgagcatgaggacctgccgggatacgcaatcaaggtgggctttaagaaagacgactcaggcgctgcgtatgcggccttctgccgagagaatgagggcatggctgggctacctgtcatccatctggtcaagcgcttcagcagggcgtacatggtggctatggacaagtaccgctcgctggatgatgttggtgggaactactgccggggcggtgagacttatgagcaacgagtcttaaacgtatcgtggcgtgtagtaaacgcggtgatagactactacgagaaaccatctgaggcacttagctggtggctggaccaagacgcgcgagctgagtttgcacacgtcgaggctcaatatattaaagaccttgcgcagactgcacgtaagattcacacgttcttctacgggctggcgtcattcgacacgcaccgggctaacgtgatggtcgataacaacgggcgcttgataatcactgacccagtgtcttggaccgcaagcgaccatcaagacgagatgcaaggaaagctgaacgcaatagctgagtgataaacgagaggccactacatctagtggtctcaaagattatttctcacaacatatagaggtgaactatgaacatctggtactgggtgtgcttatctccggtcatcttcctgatagctttcggtcttctggatgcaatcaagcgagggtctttctaatggcttgggcacttctggtcatcggctacgggttaatcctcgcagtcctcacgaaagacatcgtgaaagcacgtaaagtctaccgcttccagtatgtatcactgggccgctggactgtaagacaaccaaacgggcgctttctgcgcaacctcgcaaacgtctgggacatcgcaaccttagggagtaaactgtaatgaacaagtcatacgggattaatctggtgcactctatggacgcagaaatgaacatgttaagcctactggctaccgggtatcgtcacggaaagtcaagtcacaccacacgtcaacagcaggagcgcgaccgtgtacttcaggcacgactacgggctgagggccataagtccgaactgatgtgtctggcgtatggtggactaccaatcactgacgatggtaaacttctggtctcaggctggaaggcgataggccaacggtcaaccatcaagcacacgaccaagggtgacttcagtcatctccacgctaacccactgatatgcaagtgattatgacttaactatcactataggactcaaggtctaagactccaagtgaaagaccaaagagactttaaagtgaaagactaataacaaggaccttaagtatgagcgtcatctctattgacaaacacgacttctctgacgtgtcgaacgccattgagccgtttaacctgctggctgaccactacgggcaagaccttgcagtcaaacagcttcagcttgagcatgaggcatacactgaaggcgagcgacgtttcatcaagaaccttgagcgccagactgagcgcggggaactggcagacaatcaggtcgccaagcctctcatgcagactctggtccctaagattgcgcaagccgtcaaggagtggcatgaaggtccagacgggaagctgtcaacctctcgtcctagcgtagcgttcaccatgttgagcactgaagagaaggccgtcaaggaccgctctctgcgcatctcctgtgagtctgctgcggtcatcatactgaaggtcatcctctccaagctggtcaagcctgaagggataccgattacaccgatggcctccgcgataggtcgcacacttgaggacgaaatccgcttcggtcgcatccgtgacaaggagaaggagcacttcaagaaggcgatagctgagaacctgaacaagcgagccggggtatcctacaagaaagcctacatgcaggcagtcgaggcgtctatgcttgagcaggggcaactggctgacgcgtgggggacttggagtccgaccgaggctgtccacgtaggcatcaagatgctagagctggtcatccagtcatcgcaactggtcgagctgaagcgctacggtgctggcaatgcagcggctgacgtagagatggtccacctgtcagacttctgggtcaagaagatggcacaacgtggcttcagccttgcaggtatcgcgccagtctaccaaccttgcgtcgttccacctaagccgtggaccggggtggtgggtggtgggtactgggctaaaggtcgcaggcctctaccgctgattcgcttagggtctaaggctgcggtccagcgctacgaagacgtgtacatgcctgaagtttacgaggcggtgaacatcattcagcagactccttggaaggtaaacaagaaggtgctggaagtggtgaacatggtcgagaagctgaataacacgcctatcgctgacatccctcagatggagccgctgaagcctgaagactatgcgggtgagaccgaggaggagcttaaggcttggaagaaatctgcggctggcatctatcgacgcgagaaggcccgacagtctcgccgtgtatcgctgagcttcatcgtctcacaggctaacaagttctctcagttcaaggccatatggttcccgtacaacatggactggcgaggtcgtgtttacgcagtcccgatgttcaaccctcagggaaacgatatgcagaagggcctgctgactctggcggtaggcaagccaatcggtgcggacggcttcaaatggctgaaggtacacggtgcaaactgcgcgggtgtcgataaagtcacctttgaggagcgcatcaagtgggttgaggacaatcacgacaacatcctagcgactgctaagagtccgatggatagcattgactggtggggccagttagactctccgttctgcttcctagcgttctgctttgagtatgccggggtcatgcaccacgggctaagctactcatgctctctgcctattgcgttcgatgggtcctgctctgggattcagcacttcagtgctatgctccgtgaccacgttggtggacatgcagtcaacctgacgccaagcgggaaggttcaagacatctaccgcattgtgtcagaccgggtggaggaacagcttaaggagctgctggtcaatggcagtgacaacgaggtgaagacctttgaggacaagaagacgggtgagattactgagcgtctggtccttgggacccgtgagctggcccgtcagtggctgacctacgggatgtcacgctcggtcactaaacgctcggtaatgactctggcctacgggtcgaaggaatacgggttcgcggaccaagtgtttgaggataccgtgatgccagcgattgatagtggcaagggcgcaatgttcactgacccaagccaagcgtctcgcttcatggctaagatgatatgggacgctgtgagtgtgaccgtagttgctgcggttgacgcgatgaagtggcttcaaggtgctgccaagctgctggctgctgaagtgaaggacaagaagactggagaaatcctgaagccctgccttccggtacactgggtcacacctgatggtttcccggtctggcaggaataccgcaagaaggataccactcgtctgaacctgatgttcttagggtcattcaaccttcagcctacagtcaacaaaggcacgaagaaggagctggacaagcacaagcaggagtccggtatcagccctaactttgtacactcacaggacggcagtcacctgaggaagactgtagtccatacccaccgcaagtatggcgtgatgtccttcgcggtgattcacgacagctttgggaccatcccagcagacgctgagttcctgttcaagggagtccgcgagacgatggtcgagacctaccgagacaacgatgttctgcttgacttctacgagcagttcgaataccagcttcacgagagccagcgcgacaagttgcctgagcttccgaagaaaggtaaactgaatatcgaagacatcttgtcttcagactttgcattcgcttaataacacaggagagagacaacatgcaattcgcacaccgtgtatcaaacgtatctggcggcaacaaggtagtgaccgtaaccaaggtggctggcaagggtctggtcaaggttactatggtcccgactggaacggctaaggccaagggtatcagccagaaggagctgattcaggtaatccagtggtcacacgagaaggccctacgggaagaggcaaccaaatgacagacctacagttactggccctgtggctgggagcactcgcagtattcactttaatccaacgcagaagaggttaaccctaaactatcactataggattagactcaaggtcatgactcaaagtcgtggccttcatgattaaccctaaataaacactactggagatttaaccatatgtatcagaatactatcaacttcgagcgcatccgtgaacgtcagcagactgaaggctacattccgaagggccgcaagctgaacaagaccaagcgtggcggtggtgtcaagggtgctttccgtaacgctgaaggcaaagactcgctggttaaccaagagaagtatttcgtaggagcgtaagccatgagcagacgttggttattcgatgcgtccacgagccagtggtcatcgttaggccggacccaccgcgagatgagcgaggcaggacttgaggtcctaatggttgacctgccttactcccgaatgactctggtacgaatcattgaagcagacgggaatcctctggtatcccgcgagtttaccaaacacgaaatctttaactgtgagcaatggtgcttgcagcaactgaatgactataggagctggaaataatgacaactatcaaaaccaaccctcaccgcgctgtagattactctgagtcaggagttaagaaggcgctggctgctgctgggtctctcgaagctgaagtgaagtatgatggtgtccggttgaaccttccggtgctgcgagagggtgagacctattggctgagccgtgagtctaaacctcttccagccttggagtggatgaactctgagttaggcaatgcgtggactcaggccgactggcggtggttccttcgtcaagctggctatgaaggtatcggcctgatgattgatggcgaggtcatggtaaaaggtgttgactttaatacgtcctcaggtctcattcgaaccaagtggctcaagccaagcaatgagcactacgctgagtgctatccggggcgcggtaagaaggtcccattctgggtagcccggtcacgacttcaggttgtggtatatggcgttgtcgatatgacaaccatagcagaccagaaagccgaaggtcccatccatagcgtcacacgcctgaaggccgaagctatcgtccctctcctccagaaatacttcccggaaatcgactgggttctgtctgagtcacacacggtctatgaccttgagtcgctcaactccctgtacgaacagaagcgtctggaaggacacgagggtctggtagtcaaggacccgcttggtaaatacaagcgtggcaagaagtctggcatgtggaaaatgaagcctgaggagaccatcgacgggaccgtgtgtggcctcgtgtgggggactccgggtaaggctaacgaaggtaaggtgattggcttcgaggttctgcttgaggatggcatggtggttaatgcctgtggcctgactgaagaacagaaggacgagtttacagctaaagtcgctgaatctagcggttataccttggctggcggccctgtggttattaaggatgggaccgagaagacaaacccatacgaaggctggcagtgtgaagtcctcttcatggagcggttccctgatggctcccttcgtcatcccagcttcaagtgctggcgtggaacggaagacaacccaaccgttaagagttaactaaacgtcaacccagtggtcttcggactgctgggtttctttgctttgtgctagcaagctatcgtctgggccaccagctagaccctaagctatcactataggacaaccatcaacaacctaaggagactctatgtctaagaacttaatgttcaaccgttattccagtaccttccacctgtcaaacaacccgttcgcttgcattaagcgcaacgagaagctgggctacttcgggaaggccgttaagctgtcacctacagtctacgctctgattactcctggaaaagttgaagaggctcgcaagaagcgtgagaccaacgtacctgtggtctacaccaagtggcctcgcgttcgtctgttcgttgagtacatgaaggaggtgttctgattggatgtatttcttttcttaaagaaagacgacagttatccatacacacctgtaataaaggagttaacaatatgaacaaacttgaacaagagattatcattaagttggtagataataacgaaggtcgcccagatgatttgaatggctgcggtattttctgctataatgttccttgcgacctctgccctgcacatatcaatcaaaagataaccttaggtgaaatccgagcgatggacatacgtaagcctaaactggagaaacaagaggtaactcctacagacgaccagccttacgctaaggctatcgacgatggcgtacgcaagccgtcccactatcaggtctttgatggtgtggaatccattgagattatcgcccggtccatgactgtcagtgagttccgtggtttctgcatgggtaacgtcctgaagtatcgactcagggctggtaagaagtcagagctggcgactatggagaaggacctgaagaaggctgcattctatcaggagctgttcgacctgcataaaggtaagtgctatgctgccgagtgagtgggctgagagaaaatttgaggagacaggtaacgtagattaccttcagctctacaacttatggaaggagcgtggtctatgactgacgtagagaagaaatacatcgtggagcttgagggtcgcgttcagtccttcgaggttccggtgtacgcaaagtctcttgaagaggctaccctgaagtcccaagagtatgaggacgctgggtttgttgtcggacggattcgtcctgagacctaaactatcactgtaggacagacgtccagttagtaactttaaataggagatttacaccaatggctaaagagcaactgaagactttcaccactccggtagctggtatcgttgagccctacgcatggctgaacaaagcagacaccaagtttaatgagcgtggtgagcataaggttaatctgacattcgacctgagcaacccgaaggtccgtaagatgattgatgtcttacagaagattcacgacgatgcgtatgcgaaagcacttgcagaccacgagaagaacccacctcaggttcagcgtggcaagaagcctattgaaccacgagaaggcgacatgccgtggattgagaatggtgacggtactgttaccatgaagtttaaatgctttgcgtcttaccttaaagacggcaagtccgagcctatcgtattacggttctacgacaccgatgctaaactcatccgtgacgtcccgaatattggcgctgggtctaagctgaaggtcaagtttaaagtcctgccgttcaagtggaacgctgcgactggtgcaagcgttaagctccagcttgagtcctgccttctggtagaactgaaggagtggaaaggtgatggtgctggtggcgatggtggctggggtgatgatgaagacctcggtactggctacaaagcgtcaaccgatggtgacttcgggtctgatgacttcggtgacgatggttccgaaggaggtgatgaagatacctcaggcgactacgacttctaaatgacgctgaaagagaaactggaggcttactctaaggtttctccttctggatgctgggagtggcaacgctcccggactaaaactggttatggtcaaatagctataggtcatcagaaacaggactattctcaccgagtttcgtacagggagcacaaaggtcctatacctgatggattggttgttagacataaatgtgataacccttgctgctgtaaccctgagcaccttgaagttgggactcagaaggacaacatgcaggactgcgtgaagcggggacgtcactcgaaaccgccagtattcaaaggagaagctaatcacaagactaagctgaccgaggaagacgtagcgtttatcctgaagtccaagctgaggcctatagaacttgctaagatgtttggcgttactcagcaagctattaattggagacgcaagaatggcaagaacgattagccgagggcatcaagtaggaatatataggtctggactagaagcaaagaaccaagagtggctggagaagaacggagttaaggctgagtacgagatgtatagcatcaagtacacaataccagaatcccttcacagttattgtccagactttgtactgcccaacggaatcattgtggagaccaaaggaatcttcgcggtggaagaccgcaagaagcacctattgattagagaacagcacccagagttagacattcggttcgtgttctcaagttcccgctccaagttatacaaagggtctccgaccacgtatggcgcatggtgcgaaaagaacggctataagtatgccgataagttcatcccggttgagtggctgagagaggcgactgtacgtctgccttcaggtatactcatccctaagaagaaaggagttaagtaatgactcagaaatataaacttaaagttagttgctgcgggtggcctaaaggtactatcgttacgaaatgtgcgaaagaccctgaaccattatacggacttgttctggtggaatccactgagcgtggctactacaaacacggagcagcagggtatgacacgcagcctaacggaatgtggggggcgtgggtttcagaaggatatcttgaggaaatcttagaggataaacctcaagtccctccagcttcgagcgtaccgcctgtgactgtgaagcgtgaagtcctgaccatcaacaagattggtgtaggccagacgttcatcgtccacggtaagcctgacgaagtgtacgtgaagattagcaactcccacgtcttcaaccataagttgctccagatgcacagcacggatgctaaccgtttccaacgtcatctgaacctagtagctgtagagctggtggtgtatgatggtgagtgagactcttaggccacgactgcttgctgggtacgaggtggatgacaaagggtgctggaactggaagggtgcgactgcatccggctacggagtgattgtccttaacaggagggttgctgctaatcatgaagttggtagaaactaccagactcacagggcatcctatgaaatccaccacggccccattcaagaaggacaggtagtcaggcataagtgcgacaataagctgtgcatgaaccctgagcatctagaggtcgggacccagagggagaacattcaggacgctatcgaccgaggtcgtatggcgagtaagctgactgaggaggacgttgagttcatccggtcatcaacattaagtcaacggaggttaggtaagctgctgggcgtaagtccaactgttatctggcacattcgtaacggtaacaaatggaggcacgtttaatggctaccaaggtacaattcaagccacgtcaatcgacagaggcaatcttcgtccactgttcagcgacccaacctactatggacatcggtcgcgagactattgaaatgtggcacaagcagcagggatggctggcaatcggataccactttatcatcaaacgtgatggcactgtggaagagggtcgcccggtcaatgtcgtagggtcacacgttaaggactggaactccaagtccgtaggcgtctgccttgtagggggaatcaacgccaagggtcagtttgaagctaacttcactccagcccagatgaacgctctacgaaacaagctggctgacctgaaggtcctgtatcctcaggcagaaatcaaagcgcaccatgacgtagcgccaaaggcgtgcccaagtttcgacttacagcgctggctgtctaccaacgaacttgtaacttccgaccacggttaataaactctaaaggagaacaactcaatgattaaacttatcgaatttcttggtcgtctggtggtgcgtggttatcgtcgtgctgcggtactggaacgaaaggtagaaaagaagactgctgacggtgcggctgatgctgctgctctggctgacaagctgaccatcgcgtcactggaagctggcatgaaggcacgtcaagctgacaccaaagctgaccagttggctaagttcttcaaagactaaactatcaccttagggactggaccgtgaatccggtccctttgtccgcattattgattaaggagtgaccaatgtcatacgacgaccaaggcgagagtgtctttctgtatcacacccagtgtccagactgtgggtcctcggatgccaatggtgtttactcagacggccatcaattttgttatgcgtgtgacccttcagtagcatggaagaaaggagacatggagttgaccgagggatacacaccctcaggaggtagaaagcaagtgagcaatctgttaacgttcggtgagaacgctggacgatatgtcccactaccagcccgtagtctcagcatggagatatgcaagaagtacagctactgggtgggtaacatgggtggcaagatggttcaggtcgctgattattacgacaggtccgggaccaaggtaggacagaaagtccgagacgctgagaagaacttcacggctataggtagcgtcaagtctgacatgctgttcggctctcagctctggaacggtggcaagaagatagtcatcaccgagggcgagatagacgcactgtctgtggctcaggtgcaggacggtaagtatccggttgtctctcttccgttaggcgctaagtctgcgaagaaagctatggctgcgaaccttgagtatctcgaccagttcgaagagataatcttgatgttcgacatggatgaaccgggtcgtcaggccattgaggatgcagcaccagtattaccagcaggtcgggttaaggttgcgttcatcaacgggtacaaagacgccaacgctgcacttcaggccaaggacttcaaggccatcaccgatgctatctggaacgctaaacctttcgtcccggctggtgtggtatcagcatcaagtctgaaggaccgcacacgagaggtaatgcttaaggcagagactgaaggtctcatgttctcgtcatgcacaacactcaacgcgatgaccctaggtgcgcgagctggtgagcttatcatggtgacttcagggtcaggcatgggtaagtctacattcgttcgtcaactcctcttagagtggggcagaggtggtaaacgtgtgggtatggctatgcttgaagaggctgtagaggaaacagttcaggaccttatgggtctggacaataacgtccgtctacgtcagagcaaggaactgaagcaagccatcttagaggatggtcggtttgacgaatggtacgacaagctgttcggagacgataagttccacctgtacgattcattcgcagagtcagaggaagacaccttgttcgctaagttaggctacatggtggacggtcttgactgtgacgtcatactgctagaccacatctcaatcgttgtgtctggcatggaagataactcagatgaacgtaagaccattgaccgaatcatgactcgtctcaagaagtttgcgaagacgaagggcgtggttgtcgttgtcatatgtcacctaaagaacccagaaaaaggtaaatcgcatgaagaaggacgacctgtttcaatcactgacctacgtggctctggtgctctccgtcaactgtctgatactatcatcgcccttgagcgaaaccagcaaggtgatactcctaatattgttcaacttcgtctgctcaagtgtcgttttacgggtgacactggagtggcaggacacctcgaatacaacaagacgaccgggtggcttgaaccgattagcttcactggcagcagcggagaagaggatagcggctcgtgggaagataccgacttctaaggaggagtacattgctaagaaaacttaaagctcgataccatcggttcatgtacaaatggtggagcgatgaagcaacctgcctgtccaacattctgggagaccaaaggttcgactctaaggcatggaagaaagctaaccggaagtttatgtaccacttcttgcgtacagacttctaggtctagactcaaggtcattcacatcgagtggcctttatgattagacttataactaaaggagaagcaatatgaggacttgcagtagatgtggctctacaaaggagtccactgagttcaggaagacaaatgggtggtgcatatcctgtgttcgtgaggataataggtcgcgatatcatcgaaacaaaggtacagaggccggtgaggcgcatcgcctatctgcccgtaagtcttggcttaagaaagcctatggtctcacacttgaggaatatgacactatgttcgatagtcaaaagggcagatgcgctatatgctcagacattatcttcaagcatgggtctattgagagtaagaataatgtagcccacgttgaccattgccatgactcaggtattgttaggggattgctatgtggtacatgtaatagcgcacttggtaagttcggtgacaaggtagccgtgcttagggctgctataaagtacttggagaaatataatgtttaatctcaactcattctatggcacagatatagagactgacggtctactagacactgtgtcacagttccattgtggtgttatcattaacgctggaactcaggctactgagaaatatggtgttgcccctatgactgggctgacaggtggattcaaagagtacatagaccgcatagaatctattatggcatccactgacggtatgctggttctgcacaatggtgtgaactatgatataccagccttgaaaatactgaagaagaaatactttggtaagaacctaaatgtgaataagggtcgaattattgataccttggtgctgggccgcttgatgtatcccaacattaagttctcagacatgggagcagtgaaagctggtcgtctgccacctaagatgatgggacgccagtctcttgaggcttggggctatcgtctcggtgagatgaagggtgagtacaaacacgattacgttgccaagtgcaaggccgaaggtatcgaatataaggctggggacgaatggttgttcccgtctcaggagatgctggactataacgttcaagacgttgtggtcacactggcgttgttcaagaagttcctgactgacaagtattacttccagtctgaacagttcgctttcgaccagatttatgcgttgcgtctggaacatgatgctgcgtggacctgtgcgaagatggaacgtaacggctatccgatgaacaccgagatggtcgaaggcttatatcgtgaactcaccgtcaaacgtgcagagctgctggacaagctgcgttcgactttcggtagctggtacgcaccaaagggaggcaaggagttcttcaggcacccacggacaggtaaggaccttccgaagtatccgcgagtcgtgtatcctaaggttggtggcatctttaagaagccgaagaacaaagctcaacgcttaggtcttgaaccttgtgaacgcgatacgagagacacgatggaaggagcaccattcacgccaatcacttacgttgagtttaatccgggaagcggagaccacttagcgaaagttctgatggagcgtggctgggagcctgtggacttcactgacaccgggaaacctgtagtcgatgacgagacgttagaacacgttaagttaccagacgcagaggctcaggcttgcgtagagctggtccgtgaatatctggtggtccagaagcgcatcggtcaggctgctgaaggtaagaacgcatggttgaaacttgtaggtccagacggacgtatgcacggttcaatcaacccatgcggtgcagtaaccggacgtgcgacccatagttcaccaaacatggctcaggtcccggctaacggtgctccatatggtgagacttgccgtggtgctttcggtgcagcgtggaacaagactgatggtaagccagacccttggattcaagtgggtgttgatgcctcaggtcttgagcttcgttgtctggggaaccgagcagcaccgtttgatggtggagcctatgcgaagactgtggtcgaaggtgacatccactgggccaacgcagtaaacgctggattagcacctaacgtcccacgcgataagtcgagccacgaccatgatgctttccgtaacaacgccaagacgttcatctatgcgttcctgtatggtgcaggggccgctaagattggactgatagtcggcggtggtaagaaggaaggttcagctctcatgaagaaattcattgagggtacaccagccatcaaggacctcagggaagctgtgagtaatacgttaatctcagactctaagtgggtggacggtgagaatatcgtcaagtggaaacgacgttggttgcgtggacttgatggtcgccgtatccacatccggtcgccacactcagcactgaacgcactacttcaaggtgatggtgcggtagtctgtaagcactggattgttgagactgaacgtatgctcgaagaggccgggtatgtccacggctgggaaggagacttcgcttacatggcatgggtccatgatgaattgcagattgcagctcgtaccatggagattgccgaagatattcgcaggattgctcaacttgctatgcgtaaggtgggtgagttctataactttaaatgtgtccttgataccgaaggtaagattggaccaacgtggaaggagtgtcactaatggctattactaaacgtattcgtgtaagtttcgacctgaagatggttattaactcaaaggaagaagagaccatgtgtcgccaactggctgagatgactaaagcctacgctgagggtgagaagctggatggtcttcagttggctatggtcaaagcagcaatcgagtcaggacctgagtctgcccttgaaattgccgtcaagaaggtcatcaaggaggatctggtatacgcctttggtgattaccagttcggagtgtccaacctgcgattcgaggtcaagcaatgagtgaatacttacgggtcctagcggcccttaagtcctgcccgaagaccttccagtccaactatgtgcgcaacaacgctgcacttgtggctgaggctgcgagtcgtggacaccttagctgcctgtctatggatgggcgtaacaacggtgcgtgggagattaccgctgctggcaccaagttcctgaaccaacacggaggctgcctgtgagcgaaaagaaaatagctctggtgctggatggtgactatctggtcttctcttctatggctgctgccgaggacgagacagactggggtgatgacatctggacccttatctgtgaccatgagaaggctcgtcgtatccttgagaacaccatcgctgaaattgttaagaagcgcaaggcgtggaaagacgctaagattgtgatgtgctttactgacgataacaactggcgtaaggacgttctgcctacctataaggccaaccgtaaaggttctcgcaagcctgtaggttacaagaagttcgtagcagaagtgatggctgacccacggttcaacagcttcctgcgtcctacgcttgagggtgatgactgtatgggtatcatcgggacccgacctcagattgttggatgtgaccatgcggtgctggtgtcctgtgataaggacttcaagacaatcccgaactgtgagttcttctggttaaccactggtgaaatcctgagtcatacgactgccgaggcagactactggcacatggagcagaccattaagggtgatactacagatggctatggtggcattccggggatgggtgaggataccactcgtgcgttccttgacgagccgtactacttcgtacaggagagccgtgagcttaagaccggtaagaacaaaggacagattaagactgagtggaagaagtatcctaagcgtgaagacatgacgctgtgggactgcatggtgactctggctgctaaagctgggatgactgaagaagaacttctggtccaagctcaggtcgctcgtatttgtcgagcctccgactacgaccctaagtccaaggaggtcatactgtggacaccatccatgtaatctactgggccggacttctggccctttactgcatgtataagtggttcgggtcgaacaaccgtcctaaacactaagtctaaccgatagtcatatcctatcaatccaatagtaatccataggtgaaacactaaactatcactatagggactttaggacctaagatatgactataagatagattttagtcttaacttaaagaggagattcaagatggcgattaatgctattgaaaacgttgttaagcagttacaggaagaaagactcgatgtcccgaacatctcacagtctgccatccagttcctgcacgtactgttcaacgcaagctacgctgagaagacgggagctatcagtctcctcaagcagcagggctacagcgatgcgttcattgccgggtttatcaagggtctccagtattgctctgacactctcgactctgcgattgctatgcgtcgtgagctgaaagataccgttcagttcgattaactgtaggagggactatgtgtttcagtccaaagattagcactccgaagccttcggtccaagcacctgaaccagcacctctgagtgaggaagttgcgtcagttgacatcggggctgaatcggatgtggacaccaacgagaccaaaggtatcaaagacctgaaggtcaagaaggagtctgcacctaaagataaatcgtcagttagccgcgctatgcgagcctctggcgtcaacatggggtaagacaatgctaccatatctcaactcccgcgaaggtcgccacatgtgcgcttgtcgcctctgggaagacgggcagtctaacttcaagtcattcgaggacttcaaggctcatacttaccgtatggctgacgagttcgacggtgaagagtacacaatctacgatgtctcaggtcaaccagtagcgtatctctacatgctggctaccgcatcttggcacagaccgactcccggtctggacctttcaatagtcgctattcgtcgtgactcgcagtcctcccgcaaggttcttgagactgtcaggcacatcatagacgaagaatgcaagcgttggggtattagctggtattctcgtgtcaagcatgtttctgggtcggtagacatcgtaacaaccaagtgcgttagcatgaacaaggagattaaccgtgggtaaatcaatcagtaaggctttcaagaaagtagtaaaaggtgcgttagggaccgttggtcttggctctgatgacgcgcctaaggttgttgaggctcagaccccagcagcaccagtggaagtaccgaacgacaaagtggaggatgtggatactgaaacaaccgcatctgaggagaagaaagtgaagcgttccggtaagcgtagccttcaggtctctcgtacctctggtggcggtatttctatatgacagactgcatactgcataagggctgcgtaaataatgctggatatggtctgacgtattaacaggtaaaacatggaggcacgtagatggctaaacgtgaaggatttgctgctgaaggcgcgaagtcagtttatgatagactgaagaacggtagacagccctatgagacgcgcgctcagaactgcgctgctgtcactatcccgtcactgtttcctaaggagtccgacaactcgtctacggaatacgtgacgccgtggcaagctgtaggtgctcgctgtttgaacaacttggctgcaaagctaatgttggcattattccctcagtcaccgtggatgcgacttacagtctccgaatatgaggccaagaccttgagtaatgactcagaggctgctgctcgtgttgacgaagggctggctatggtcgagcgtgtgttgatggcctacatggagactaacagtttccgtgtcccattgttcgaagctctgaagcagcttatcgtctcaggtaactgtctgctctacattccagagcctgaacagggaacctacagtcctatgcgaatgtaccgcttagtgtcctacgttgttcaacgtgatgctttcggtaacatcttgcagattgtgactctcgacaaggtagcgtttagtgctctaccggaagacgtgaagtctcaactcaacgcagacgactatgagcctgataccgagctggaagtgtatacgcacatttaccgtcaggacgacgagtatctacgctatgaggaagtggaaggcattgaggtagcagggaccgaaggttcttacccactgactgcctgtccgtacatcccggtacgaatggttcgactggatggtgaagactatggtcgttcttactgcgaggagtatctgggagacctgaactcgctggagacgattacagaagctatcaccaaaatggctaaggtagcctccaaggtggtgggcctcgtcaacccgaacggtatcacgcaacctcgtcgtctgaataaggcggctacaggtgagttcgtggctggtcgcgttgaggacatcaacttcctgcaactgacgaaaggtcaggactttacgattgccaagtcggtggctgacgctatcgagcaacgtttaggctgggccttccttcttaatagtgctgttcagcgtaatgccgagcgagtcactgctgaagagattcgttatgttgctggcgaactggaggcgaccttaggtggcgtgtactcagtacagtcacaagagcttcagttacctatcgtccgtgtgctgatgaaccagcttcagtctgctggcatgattcctgaccttccgaaagaagcggtagagcctacggtatccactggtctagaagcgttaggtcgtggtcaggacttagagaagctaactcaggcagtcaacatgatgaccggtcttcagcagctctctcaggacccagacattaacttgccgaccctgaagctgcgactgctgaatgccttaggcattgatactgctggtctgcttctgactcaggacgagaagatgcaacgtattgctgaacaatccgctcaaggagctgtggtcaacggtgcgtctgctgctggtgcaaacatgggtgctgctgtaggtcagggagctggtgaggacatggctcaagcctaaactatcactataggaacaacacaacttgagtgagtgaacgcatggccagccgtaactgactggcaggttgttgtgtttcctattaactaccaaaggagaatgactcaatgtctcaatcagtttatgccgagttcggcgttagctctaatgcaatcactggttccgttgaggacctgaacgaacaccagaagtctatgcttgaacaggacgtagctgttcgtgatggcgatgacgctattaccttcaagcaactggaagctgaaaatgaagaggcgaccgaagaagacgaaaacgtcgaagagactgaaggtgaagaagaccacgagtcagatgacgaagcgtctgagaccgatggtgctcagcctgagttcatcgaactgggtgatgcaccaaaagagctgaccgaaagtgtaacagctctggatgaaaacgaagctgcattcgatgacatggtgtcttctgctgtagaagctggcaaggtcactgctgacgaaattaccgctatcaaggctgaatacgccaaggacggtaagctgtctgacgcatcctacgctaagttgcaggaagcaggttataccaagcgtttcgtagattcgtttgtccgtggtcaggaagctctggctgaacagtatgctgctggtgtggttcgctatgctggtggtgctgaacagtttaatcgcatcctgtcacaccttgagtccaacgacccgtcaactcgtgaggcactggaagctgctatcgttcgtaaggacattgcgactaccaaagctctgctgaatctggctggcaagactctgggtaaagctgtgggtgttaaacctcagcgtaccatcaccactcaggctaaacctgtggtcgcacctaaggctcctcagaccgaagcattcagctctaaggctgacatgattaaggctatgagtgacccgcgatacctgcgtgacgctaagtacacgatggaagttcgcgctaaggtagctgcatcaagcctgtagttgactaaactatcactatagggagaccaagagactctgaaaggaagagactcaatgtttccctattacttcagtccatacggattgggcgtacagtaagtaataaactttatctttcaattgaataggagaattatcatatggcaaacgttccgggtcagaaaattggtacagaccaaggtaaaggcaaatccagttccgacgctctggcgttgttcctgaaggtatttgctggtgaagtcctgaccgcattcactcgccgctctgtaactgccgacaagcatattgtccgtaccattcagaacggtaagtctgctcagttcccggtcatgggtcgcacctctggtgtgtatctggctccgggtgagcgactgtccgataagcgtaaaggtatcaaacataccgagaaagtgattaccattgatggtctgctgacttccgatgtgatgattttcgacattgaagacgccatgaaccactacgatgtggctggcgagtattccaaccagctcggcgaatctctggctattgctgctgatggtgcggtactggctgagatggcgagtctgtgtaacctcccggctgcatccaacgagaatattgctggtctgggcactgcgtccgtacttgaagtaggcaagaaagctgacctcaacaccccggctaaactgggtgaagcaatcatcggtcaattgacaattgctcgtgcgaagttgacctccaactacgttcctgctggcgatcgttacttctacaccacgccggacaactactccgcgattctggcagccctgatgccgaacgctgctaactacgctgcgctgattgaccctgagacgggcaacatccgtaacgtaatgggcttcgttgtggttgaggttcctcacctgacgcagggtggtgctggcgaaactcgtggtgacgatggtatctccattgcttccggtcagaaacacgccttcccagctacttctactggtgatgttaaagttgctctggacaacgttgtgggcctgttctctcaccgttctgctgtgggtactgtgaagctgcgtgacttggcgctggaacgtgaccgtgacgtcgatgctcagggcgacctgattgttggtaagtacgctatgggtcacggtggtctgcgtcctgaagcggctggcgcactggttttcagcccagcggcgtaagcacctttagccaacctaacgtcgctacagtagcggctgcacctgaagaggagactctaactcctcaacagaaagctgcgcgtactcgtgctgcgaacagggccgctaaactggctgagtccaacaactaattgaaaccccttgggtgccttcgggtgcttgaggggttttttgcttaaagtgagaggagacttatggctcaatacattccactgaacgctaacgatgacttagatgccatcaacgatatgttagctgctatcggtgaaccagcagtcctacagcttgacgaagggaacgctgacgtctcgaatgctcagcgtatcctgcatcgtgtaaatcgtcaggtccaagctaaaggctggaactttaacatcaacgaagctgccgtcctgacacctgatgtccaagacaataggattagattcctaccgtcttatctccgggtcatgactgctggtgctaccagttactacagcaacatgggaggatacctttatgacctgtccactcagtccacgaccttcactggtccaattacagttgaactggtagagatgaaaccgttcgctgagatgcctgtggtcttccgtgattacatcgtgaccaaggcaagccgtgagttcaacgctaagttcttcggtagcccagagtctgaactatatcttcgtgagcaggaagcagaactctaccagcaggtgatggagtacgagatggacactggtcgctacaacatgatgtctgacatagggagggactaatggcctaccattacctgaagattgaccctgagttctttgagcctgttatctcaggactaaagactgctgagctgagactcaacgacagggactataaggttggcgactggctaatcctgcgcgagtggcagaacggctacacagggcagcaggtagcacgaaaggtcgttcacatagctgaggtagacttcgtgtctcccggatacgttctaatgagcatcatctaaaggagggcttatgccgctttacacacaaagtatcaagaacctaaagggtggcatgagccaacagcctgacatcctcaggttccaagaccaagggtcacttcaggtaaacgcttggtcatctgaaagcgaggggctacagaagcgcccacctacagtctggaaacgtcgagtagctaacgaggctgacatccctgataacgctaagttccacctgattaaccgtgacgagaacgagcaatactacgttgtgttcaccggccagacgataaaagtattcggacttgatggaacagaatacgttgtcaacggagggtcaacctacctatcgtccgcaaaccctcaggcagacttcagggtggtgacggtcgcagactatacgttcatcgtcaacagacgtgtagttgtttcagcaggtacagcggttagccaccccggttatgacatgaagcatcgcgctctgattaacatacgtggtggacaatatgggcgcacccttaccgtctcaattaatggtggaccagctgtatcccatgtccttccgaatggtagtaatgctgagactgaccctccaaaggtagatgcccagaacataggcttcgagcttcgagcacttctggtagcagcttatccaacctacacgttcaacttagggtctggatacattgagattattcctcctgatggtaccaacattagcagcgtggagacagcggatggttattctaaccagttaatcaacgcagtgttggacaccgtacagagtgtgagtaagttaccactagccgcacctgacggctacattatccgaatccaaggcgagacgaacagttctgctgacgaatacttcgtaaggtacgatgcctctcgtaagacttggcgggagactgtggagccgggagtggtaacgggtctggaaccggggactatgccacatggtctaatcagaaagtctgacgggagctttgactttacgtctctggattgggcaggacgtggcgcaggcaatgatgatactaaccctatgcctagctttgtgggtggaactatcaatgacgtgttcttctaccgaaacagactgggattcctgtcttccgagaacatcatcctgtcacgctcagcaagctacttctcgttcttccctaagagtgtagcgacattaagtgatgacgaccccattgatgtagccgtgagtcacccacgaatctcaatcctgaagtatgccgtaccgttcaatgaacagctccttctgtggtctgacgaggttcagttcgtgatgacaagctctggggtacttacctcaaagtccatccagcttgacgtaggatcagagttcgctgtaagcgatgatgcccgaccttacgctgttggacgctctgtcttctttagtgctcctcgtgggacgttcaccagcatcaaccgatactttgcgatggctgatgtaacggacgttaaggacgctgacgatgtgactgggcacgtattgtccctcatccctaacggagtgttcgatatacaagggtcctcgactgagaacttcatagcagtgactaccagcggtgcaaggtctaaggtctacatctacaagttcctgttcaaggagggcgtgcaacttcaggcatcttggggcatctgggactttggcgagtacggagactgtaaggttctggcaactgcttgtatcgggtccaccatgtatctggttcgtaagtcgaccaagggtattgactttgagcatctgaccttcatcaaggactccacggatattcaaggtgagccttatcgtattcacgctgatgccaaggttgactacatcattccagccagtggttacgacatacagaagaatcagacaacgttcgacatcactcaggcatacggtaagattccagccaacggtatctaccagattgtcgccgctgacggtcgctgtgtacgactcccagagcaggacttcatgtttgagcctaacgtagctatcaatggtaactggggaggactgagggtcttcataggccgcgtcttcaagatgacctatgagttctctaagttcctcatcaagcaggaggaccagaacggtacgcagactgtggacacagggcgtctacagcttcgcagggcatggattaactatcaggatacaggcgctatgatactgaaggttaagactccagcgcgtgagtttgagaacactctcaacggctataagctgggccagcagaccatcgggtctgtgagcattgggtccgggcagtttaggttccctatgaacggcgacgccacccacacgactctgacactagagtccgactatcctaccccagtgtccatcgtagggtgtggctgggaggcttcatacgcgcgtaaagcgaagtctatctaacttactgattggcctatagattcaccttaactatcactatagggactataggccctttaagttataatactttaagaggagactttatgtatattcgtaaagctacggaaccggatgtccactactttatgtggcatctttcagcagatgacgttaaggagtgcaaagcaaactacgggtcaaccgtgggtctctctgaaagactgcttaagcatctaactccgtcatctgtggtcttaactaacggtgtaggcgaagtgtttgcctatggtggaaaccaaggagataacgtatggttcttgacttccggtcttgtctacaagctgagacctaaagagaagctagagttcgttcagcgaatctctgagtacagggacttaatgttagaccaatacgggaccatctggaactacgtgtggtcaggcaataagtctcacattaaattcttgaagttactaggcgctaggtttcacgatgagtggaccacaagtccggtaactggtgagcgatttcaattattcacaatctctaaggaggacgtatgtgcgagccgactagcataggcatgggtatcatggctgtagccggggctactatgtccgcatctcaacaggccaaggctgagggtgctgctatcgacgctcagaacagacaggctcaggaaatggttaagcagatgaactactctgacgccaacctgaggatgcaggagcgagacctgaaggaacagcagatgactgaactgacagagaccactctcaatggtatccgcaatcagggtatggtccgagctgcggtagctgagtcaggtctggaaggtaactctatggacaggattgaacgtcaggtcgagggagatacagtcaaggagagagcagggattaccgaaagttacaaccgcgactatgcggctatcttcgggaaccgtatcgccaacattgagaacaccaagtctgctatccgcggtcaaggtaaaatcatcaagaccagcccactggctcatgcacttaatgttgctaacgccgggatgcaagggtacgctgctggtaagtcaatctctggggcatcaagctctggtggtgctgcaccgattagtgctgctaaaggcacacctacaggtcatagctaagaggaggactaatggctagtaatattgaatcagctctggctaatcggactatgggtcgtggcagagcgcctggtaaaactatcgccgtcaactatcaagcagccaacgttcaggctccgactggtgactctggtctagctcgtgcgttaaccaacttcgttgagtctgggactggattatacaagcagttcaaagacgaggagaagaccagagctgatgagcggtctaacgagattatccgtaagttgacacctcagcaaagacgtgaggctatccagaacgggacactgctatatcaggacgacccttacgctatggaagcacttcgagtcaagacgggccgtaacgctgcctttgcggtggatgacgagattaacgttaagattcagaacggtgagttccgtacacgtcaggacatggaagagtatcgccaccagcgacttcaggatgctgctaagtcctatgctgaagaggcaggtattaaccctaccgacgagttcttccagcgtggatttaacgataacatcactgaccgaaacatcgctatctacgggtctttcaataagtatttcagcaagcagtctgaagagacagcaatgttgaacactcgtattgagctgaactcgttccttaacgatggggacctgatgcgttcgcctgagtctggaaagaccttcatggcctaccttcgggatggactgacgactgctgctataccttcggaccagagagcacgagaggtcatcacccagacggtccgtgacgcaatccagaagtcaggaggctcaaacttcctacagcaagtccgtggcgagcgtatcacccttaatggtgttgacgctaccatcgaagaggttgtaggacctgacgtcttcaatgctgctatggttgaggcccaaggtactgagtataaactggtggctaagtatcaggaagacttggcgttaggagttcagtctgcgattcttcaggacgacccaaccatcggtcttgcccagattcagaaactcaaggagcagaacaaccagcttcaacccggcgaagaactcactcctcagcgtcagatgcttattaatgccgaagccagcttacttgaagcggtaaaacgtaagtctgctgaacaggcgaaggagaacactaagttaatccagactcagaacaagcaactggtcattgaccaagtgtatcagcgacgtctggctggggacaacgtgtccaccaactatgaggaccttccggtatctgaagctacaggagagttcaagcgttcagacatgaacaactatgcgtctgccaagctacagcagattgaccagatggacatccctgaggctgctaaagatgctcagaaggtggcattgttaagagctgacactaacaacggtcctttccgtaatgccttccagacgcttactcaggacgctgctggtgagtggcaagctgcggtcatccgtggacagtacgacccagacaagatgaaacgcttcgagtctcttcgtcgtgcctacactcaggacccttcaagtttcgctgctctgtatcctgaccaagctcagctgttctctacgttcgaccagatggacaagatgggtcttgaccctcagacgatgattgaagctgataagcaagctgcaagtcaaagccgtgagatgcgcatggaatcagacaaggcgtggcaggagttgaagaacgactccaagaacacccagttgtctcgcctcccaacgtctctggattcaagtgctcgtaaggtctgggactcatggtactatcgtacaggtaacgctgatgctgcaactcagcagactcaacgctggctgaacgagaacaccgtaacgttccagtctgaaggttctgacggtaagtcaatcggcatggtatccaagcaccagcttatggtcggggataaccctgagtcgtggcaggtaggtcgagacattatcgacaccgcccgtaagcagctcattaaggccaacccttgggtagtgaactctcagttgtccgttgttgaacagaacggctctatcttcctccaagacgctacaggtaccattcgtattcgctacgataaggaacttgtaggtaaactctaccgcgaacaacagcagaaggcacaagatgccgcatatgctcaggcagaacgtgacgctaacaagcgagcgcgtatcgtcgggactaaagctgctggtgataaacgtcgagctgaccgagaggccaacatcgagaagcgcggtgggatgtacaatgacgtctcactggagggtatcgcaaacgtattaattggtaaggagtaacataatggcgacacgtggagtaaggaattcaaaccccgggaacctccgtaagtccaaagaccagtgggaaggtgctataggtgatgatggtgaatttgttatcttcgacagccctgaatccggggtccgagccttagcaaaaaaccttcaaagctacggtcgccaaggctacgactcaatcgagaagattatcagccgctgggcaccacctaatgagaacgacactcagtcatacatcaactctgttgtggctgctactggcattccagcgacccagagtctcgacctgacgaaccctgacgtcctcgcctctctgtctgaggctatcggctaccacgagacaggctcccggtacgaccctgaagtctatcagaagggagtcgcacgggcactcaacggtatcaccccaaagaccccaccagtaagcgctaacgtatttgacgctctcacggagggcttgaaggctaaacctaaagtagctctgggcgagaaccttccgaccgctgctggtctaaacattgagggtcaagcacctgaagctcccaacgaatcgttcggtgagatgttctataaggctactggagagaccatgcaggagcgagaggatcgctctacgtggttcggtttcggtgctgctgcagaagctgaagtgaagaactctatggtcggcgtggctatccgagctggtcagactgaggattcactggatgtcattggtgatgtgttcaacccgaccagatggaacaaccataagtggtcgcgtgaggagctggaccagattcgtaacgctggggttctgcctcagtattacggagtcattactggtggctctcctcagaacctgaccgagcttattaacttggcgcttgagaaccagaagttggaccaagagaaggccaaggctgggactggcgctcagttagctgctggtgttattggtgctggcgtggaccctctgacatacgttcctattgctggacaggttggtaaaggcgctaagctggtcaataagatgttcaccgtggctgctcaatctggagcactggctggtgtgtctgagatggcccgtacctcagtggctggtggtgatgctcatgtggcggaagctatccttggtggtgctctcttcggtggtggtatgactgctatcgctgatggactaggcagagccttaggtcgcaacactaatgagttcgctggcccagctacacgtctggaagctcgtgagaccgctcgtaacgttgatggtcaggacctgtctcgtctccctattcaggaaggtgagcagacctttagtcatcaaggcgttaagttcgctgacgttccgaacgagtcgggtagtgtacgacttgaagatggttcaatcctgattggtgagaaccctctgaaccctaagacacgtcaggtctttgatgaagtgattgagcctgaacgtgctgctgctggtgtgaaccttggtgggctgactgagattggcctgaagcttcttcggtccgagaaccctgagattcgtggagtcgctgctgacttagtgcgttcaccgactggtatgcagtcaggggcctcaggtaaaatcgggaccactgcgtcagacgtattcgagagacttcgtgctgtggaccatcggttctacaacgacatcgacgatgcggttactgaggcgctcaaggacccatacttccagacagcattctggcgagactctggcgcattccgtcaggacatctaccaacgtgtgtctatggctatagaagatggtagcgggaacctgaagtctgaactgactccgggagaactgaaagtctacgacctgctgaagaaccagtttgacgccaagcgtgagatgatggagaacccagcgatgtttggtcgtccagacgctaagtctatctttccgggtagtcgcttcaagggaacctacgtcccgcatgtgtatagcaaccagatgaaggagctgtacatcaaggagcttggaagtccagaggcactacaggaggccatcaagaagtcatggttgaccagctatgcgtctcggcctgaagtcaagaaacgtgtggacgaggcactcttagaggctgaccctactctgactccagagggacttgctgctgcggtcgataagtacgccaacgataaggcttacggtatctctcacaccgagcagttcgaacgttcatccgtaatggaagagaacatcaacggtctggtgggtcttgagaacaacagcttccttgaggctcgtaacctgttcgatagcgatatgtcaatcgttctgcctaacggtcagaccttcagtgtcaacaacctgcgtgagtgggacatggacaagattgtcccggcctacaaccgtcgagttaatggtgacattgctatcatggctggtacaggcaagaccacgaaggacatgaaggacttagttgagaccatgatgaacaaggctggtgatgatggcaagttgaaaggtgaggtctcgaccttacgagacaccttgaagattctcactggtcgtgctagacgtgatggtgctgacgatgctgccttcgctacagtgatgcgcacaatgacagacctatcgttcttcgctaagaatgcctacatgggtgttcagaacttaacggagattggcggtatgctggctcgtggcaacgttcgtgcaatgctgcatggagtcccgatgttccgtgacctagccttccgtaacaagaaggtcggggcctcagagattaaggacctgcacaatgttatcttcggtaaagaactggatgactcaatccgtccgtctaaacaggacgtcattgaccgtctgcgagcttacagtgacctcggtcgtggtacagctacagctcttgggactgccaagtattacactggtgaacttgcagtacgctctccgttcactaaagtcctgaacggtacgactaactacctgcttgatgctggacgtcagggcttcttgtctgacatagtggagcacagcctgaccggaagtaagcgtaagtttgatgaccgctggttgaagaccgctggtatctccgctgaccagtggaagggcattaagtccctcatccgtgagtcagtgactcgtggtccagacgggaagtacaccatcaaggataagaaggcgttcagtcaggacccaagggctatggacctctggcgcatgggtgacaccatcgctgatgagaccctcctccgtcctcacaagctgagcaacatggatgcaaaggcttatggaccgctggctaagactgtcttgcagtttaagaacttcgtcatcaagtctatcaacggtcgtacaatgcggacctactacaacgccaccaagaacaaccgagctattgacgctgcgctgtccacggtgatgtctatgggtctggctggtatgtactacatggctcaggcgcacatcaaggcctacgctatgcaggatggccgcgaccgtgagtacctgaagcaggcgcttaaccctacgatgattggctatgcggctctgtcccgtagctcacacttgggtggcccactcggggtcgctaacattctaggtggcatcgctgggtatgaggacactaagcttctccgttcgtctatcctccctcgttcacctacagagaagcctgaacgtgccatcccgtatggtgcggctacaagtgaccctgtgatgaatgtcgtcggtaacttcttggagcaggttccagctttcggctatgctgctaacgttggtgcttcggcttacaacttggctggctacctaaaggccgatactcgtgtcaacgagcgagactatatgacaggtatgtataataccttccgagaactagtcccgaacgacccaattactcagaagctactgcttgggaccttcgaggagcaaggcatccacatcaaagactaaactatcactataggaaacgggacactaacataggtccctcttatgtcaaactaaaggaggccaaatgtcaggcactttaactcagttccctacagggagcactcagtataaaattaacttcgagtacctagctcgtgcattcgtggtcgtgactttggtcaactcttctgataactctcagaaccgtgtactgactgtgggcaatgactacacgttccttaaccctacgacaatctatgtaactgctaaccaagccggttatgacattatacagattcaccgtgagactactacagaacttatcgttgacttccgtgatggctcagtcctgactgctagtgatttaactaacgctgagcttcaggctgtccatatcgcagaagagggtaaggaccagactattgaacggggtcgacagtatgctgaagctgctggaaaagaatatgagaacgctaagtctgagcgcgaagctattgaggacattgtttcaacttctggctgggactctaagttgcgttctgatttagcaggggctgatggatacacattagtgcctactgttgcgcctaagaactcagtaacaagagtgcccattacgacgttcccttcgtataataattcagctattgagcaagcaatgtatgactcggtgcagactctgggatatgcatacatccccggcctaggcgcggaatacactaagtatacaatctcaaacactatatcaccctcagtagatttaacaggtgcgcgcgtgattgtagacgatatggtttggatagattcaaactatgacaactactcattctttaaatcgttaaactttgagggcaagtgtaagtttactttcagaaacggattgtttgggatgactggtggtgaggttgaagccttacctaacgtcggacgactaaatgaatctccagtatccatctcccctatatcgttcgatgatacgtatgtacgtattctacagagtgacctagatactttctccaccggggttaaaggagcttctaatgattactcctgtgagtttgcagttgaagctggtaagtatgctggattgtttaccggaataaatattggtgagacgataacagggcatataggagcagcgcacggacaggaaaaagctgaatcgacaggtgtcttactccgtggagaactaggatggattctattcgacggatttagtaatgggagtgagtggcgttacagggttaagaagaaaggcgaatcaatggtaaatggtgcgtcaatttccgtacctgagtctggaatgcttaaatcgtactctccgtccaatgctacagttggtattagccttacagcagcggacagattcaactttattgtcaatggggtaagtttgaccccaacattcacatcactagtaggatccatttatgagataggattcgttagttcgaaccaaactactatgatgcagagagtaacaggcctgaatctctacacatcaaagcgaggagtctttgggcatgctcctcttcacatcttgatacgtggagattctaccgcagaaggattcatctctacttttgacaagtatctaccgggtcttctcgacggctccatgggtacacgcagtttatcaattactaacaaggctattgctggtgcgttcatgcgtcagcagcttgacgaccttaaggctgaaggcgctggacaggcatatatggtaatcatggttggtggaactaatgaagggcaagctaactacagtcctgacgcgttcggcgcaatggttaaggagtttgctgattggtgcatttctaatggtagagttcctgtctgggttgagccgtggatgtggtattcgaagacattcgtaggaggtgcaggacaagactctagtaactacgagaatgctgcacaattgcgagagtcaggtaaaagggctatggcttcttatggagacctcggtatatgcgttccgacgacacacatactgccagcacctatgcctgagtatgtaacatctggtgttgctccactattacgtgatgatattcaccaagatgagttagggtataaactctatgccgaagccattgcgtccgcgatagtaggctggtcgtccaaggtatcatctaggccacgtccagcatggagcgaatggtctcgcaatacagcttcaataacgtacccatccatagtaaccactaatagtattaacgtatctatggacatcactggcttctcaaatggacaggttgtacttaacctaccacgagggtgccgtccagtggttactacggtagcgactgttacacacactactgataacatcaactatgctgctggtttcgctctaatagctcctaatggcgacgtgactgtgcaggggcttaagtcgacagaaggtcgcataactattgtagcaaattggtaaataactggaggccttatgattgagttagacttcaagaatgaagttcttaaggcctcccctatcgttgggaccgctgcggctgatggtgccagtcggttcttctttggactcacactgaacgaatggttctacgttgcagctattgcgtacaccgttgtccagattggtgtgctggtctacaaaacgattaaagggggaggaaagtcatgacacaaatggacttagagaagttcctgttaatgctagatacagagcgtgcccgtctcatgctgcaagacctgcgggatgacactaagcgttcacctcagctctacaacgccattgagaagctactagctcgtcacaactttgtgttaagcaaggtgtctgtggacgagaagacgctggctgatatggaggccctgaacgcagagtacgataaggtgctttcagctactgaggataatgacaccgggtatggtgttcaataagtgttagactcaaggtcatcgtcaggtggcctttatgattaacactaaggaggttacatgaaagattcatacataagtggcggttactggaaggttactcgtaacggtaaggttcatggagttcatagattactatgggaggaagcctacggtactatcccagatggttacgtcatagaccacattgataggaatcctatgaataacgaactgtcaaaccttaggtgcatacctaaaggcgcaaacaaggctaacacggtatcctctagggaactacctaaaggcgtatactctaggtttgctaaacgtcaaggtgtaactgtgtactatggtgacattaggatgggaggtaagaaagaaactcatgcgcctactaagaatctgaaggaagtcgtggaatgggctaagtcaactcatagcagaatgctaaaggagacatatggtatttcaaatgtttaagagagtggctccgtggttacttgcagcagtgatgtttgctggtggctaccacaccgctaacaataagtgggaggctaaggtcaatgcagaatacacctcgaatcttaaggcatcggaggatacaaggcttgctgtccaagctgaagtcaacaaagtgtcaaagcggtttcaggacgaaatgtcctcgctggaaggcagcactgataggattattgctgaccttcagtctgacaataagcggctgcgcatccgagtcaaacctacgagtggagccacgcaaagtgacggtcgatgcgtcattgatggttacgccgaacttgacgaacgagatgctaaacgtcttatcgccatcggagtgaaaggagacaaatggattaaggcacttcaggacactgtgagagccttacagcaagataaggaggggacgcattgagtaaagacttagtggcgcgtcaggcgctaatgactgcccgtatgaaggcagacttcgtgttcttcctgttcgtcctgtggaaagctctgtcactaccagtcccgactcgctgtcagattgacatggcgaagaaactatcggctggggacaacaggcgtttcatcctacaggcgttccgtggtatcgggaagtccttcattacgtgtgccttcgtggtctggaagctatggaacaacccagacttgaagttcatgattgtgtcggcctcaaaggaacgagccgatgcgaactccatattcatcaagcgaatcatcgacctcatgcctcagcttcaggaactcaaacctaagcagggacagagggacgcggttatcagcttcgacgttgggccagccaagccggaccactcaccttcggttaagtccgttggtatcactggtcagctgactggtagtcgtgctgacatcctgattgccgatgacgtggaggttccaaacaactctgcgactcaggctgcacgagaccgtctgtcagagcttgtgaaagagttcgacgctatcctgaagccgggaggtacaatcatctatctgggtactcctcagaacgagatgaccctgtatcgtgagcttgaaggccgtgggtataccactactatctggcctgctcgttatcctcgtgataagaaggactggcagtcttacggcgaccgtctggctcctatgcttcaggcagaactggaagaggaccctgagtccttctactggcgtccgaccgatgaagtacgattcgatgatacggacctgaaggaacgtgagctgtcctatggtaaagctggcttcgctctacagttcatgcttaacccgaacctgagtgatgctgagaagtaccctctgaagctccgtgaccttatcgtagccgacttggacccagcgtccagcccaatggtctaccaatggctgccaaaccctcagaacaagcgtgaggacgttcctaacgttggactcatgggtgactcataccacacgtatcagactgtaggttctgccttcagttcgtacacccagaagattctggtcattgaccctagtggtcgtggtaaggatgaaactggttatgcggtactgtaccagctcaacggatacatcttcgctatggaagttggtggtatgcgaggtggctatgaagactctacgctggaagccttggctaagattggtcgtaagtggaaggtcaacgaatacgtcattgagggtaacttcggtgatggtatgtaccttgagctattcaagcctgtagcggcacgtatccaccctgcggctgtaactgaagtgaagagtaagggtcagaaagaactacgcatctgtgacgttctggagcctatcatggggtctcacaggcttatcgttaacgctgctgctatcgtccaagactaccagtcagcctctgataaggatggtgtgcgtaaccctatctactctctcttctaccagatgacccgtatatctcgtgaacgtggagccttggcacacgatgaccgacttgatgcgctggctatcggtgtacagttcttcgttgagtctatggctaaggatgccaacaaaggcgaacgtgaagtcactgaggagtggctggaggaacagatggaggacccacggaaaggcttcgagtccatccacactgagttctgggacaatggggtccgggtaactcatgatacggacgacgagctgggactagggtcatacgttacgttccactagctgaatgaataactatgggtgaaagctgcatgaatacgcggttagtaacctatagttactaccagtctaacctactgttttataagaagtttggacttaactatcactataggaaagaccaatggttacttatagtattactgtagtgaatatacatatgcagactttatgcaagaccttaggaggcagactccgagttcttacctaaggcttgcaccgatggaaggaggtgatattaatcataatccctccaatacagatagtcaccgaccatagatacaggaggtatgtagcatatggcaaagaccaaagctgtacttaaagctctggcgaccaatcgagctacatacaggtttcttgctgctgttctacttgctgctggcgttactgctggaagtaagtgggtcgggtgggtcgagactctcgtatgttctctggtctctcagtgtaattaacgcaatcatggtaacgattcatgagtggaagacctaaggtcagttcatagctgacgctactctactgaccttagctactgtagtcaaggactttaggtaacaccttaagagaagctcacttagggtcatcctacttactggtctaccctagtgtcgcctgacctacggtccttgacctacagtggctgtggcctacagtagggacgatgagttttggaccaaaagtttgagaccaca